European Patent Application EP 4 230 724 A1, published August 23, 2023. Title: Medium for production of extracellular vesicles. Applicant: FUJIFILM Wako Pure Chemical Corporation. The sequence listing filed with the application follows.

SEQUENCE LISTING (2 sequences)

SEQ ID NO: 1 - DNA, 22 bp, Artificial Sequence
  oligonucleotide primer
attgctgggatcactggagcac

SEQ ID NO: 2 - DNA, 24 bp, Artificial Sequence
  oligonucleotide primer
cctggtttcccactttcacccttg